European Patent Specification EP 3 425 047 B1, published April 24, 2024. Title: New Polyphosphate-dependent glucokinase and method for preparing glucose 6-phosphate using the same. Applicant: CJ CHEILJEDANG CORPORATION. The sequence listing filed with the application follows.

SEQUENCE LISTING (4 sequences)

SEQ ID NO: 1 - DNA, 762 bp, Anaerolinea thermophila
atggggaggcagggcatggaaattttagggattgatatcggaggatccggcatcaaaggggctccggtggatgtagaaaccggccagttaaccgccgagcgataccgcttacccacccccgaaaatgccttacctgaagaagtggctctggtagttgcccaaattgtcgaacactttcagtggaaaggtcgtgtaggggcaggatttcctgctgccatcaagcacggcgtggcacagacggccgcaaacatccaccctacatggattggacttcatgctggcaaccttttcagcgaaaaatgcggatgtcctgtctcagtgttgaatgatgcggatgctgccggactggcggaaatgatctttggggcaggaaaaggccagaaaggggtggtgctgatgattaccattggcactggcatcgggacagccctgttcaccgatgggatattggtccctaataccgagttgggacatattgaaattcggggcaaagatgccgaacagcgctcttcggaagccgcccgccagcggaaggattggacctggcaacaatgggcaaagcgtctgaatgagcatttggagcgcctggaagccctgttctggcccgatttattcatccttggtggaggggcagtaaaaaatcatgaaaagttcttcccttatctaaaactgcgtactccctttgttgcagcaaaattggggaatctggctgggattgtaggcgcagcgtggtatgctcacacccaggaaacgcaagcctga

SEQ ID NO: 2 - protein, 253 aa, Anaerolinea thermophila
MGRQGMEILGIDIGGSGIKGAPVDVETGQLTAERYRLPTPENALPEEVALVVAQIVEHFQWKGRVGAGFPAAIKHGVAQTAANIHPTWIGLHAGNLFSEKCGCPVSVLNDADAAGLAEMIFGAGKGQKGVVLMITIGTGIGTALFTDGILVPNTELGHIEIRGKDAEQRSSEAARQRKDWTWQQWAKRLNEHLERLEALFWPDLFILGGGAVKNHEKFFPYLKLRTPFVAAKLGNLAGIVGAAWYAHTQETQA

SEQ ID NO: 3 - DNA, 34 bp, Artificial Sequence
  Primer
caccatatggggaggcagggcatggaaattttag

SEQ ID NO: 4 - DNA, 29 bp, Artificial Sequence
  Primer
caaactcgagggcttgcgtttcctgggtg